European Patent Application EP 4 549 580 A1, published May 7, 2025. Title: RNA 염기서열 분석을 위한 라이브러리 제작 방법. Applicant: 주식회사 제노헬릭스. Application KR. The sequence listing filed with the application follows.

SEQUENCE LISTING (8 sequences)

SEQ ID NO: 1 - DNA, 33 bp, synthetic construct
  source 1..33: mol_type = other DNA
tggaattctcgggtgccaaggaactccagtcac

SEQ ID NO: 2 - DNA, 55 bp, synthetic construct
  source 1..55: mol_type = other DNA
gatcgtcggactgtagaactctgaacgtgtagatctcggtggtcgccgtatcatt

SEQ ID NO: 3 - DNA, 52 bp, synthetic construct
  source 1..52: mol_type = other DNA
caagcagaagacggcatacgagatctgatcgtgactggagttccttggcacc

SEQ ID NO: 4 - DNA, 12 bp, synthetic construct
  source 1..12: mol_type = other DNA
tccgacgatctn

SEQ ID NO: 5 - DNA, 22 bp, synthetic construct
  source 1..22: mol_type = other DNA
aatgatacggcgaccaccgaga

SEQ ID NO: 6 - DNA, 24 bp, synthetic construct
  source 1..24: mol_type = other DNA
caagcagaagacggcatacgagat

SEQ ID NO: 7 - DNA, 20 bp, synthetic construct
  source 1..20: mol_type = other DNA
tattgcacttgtcccggcct

SEQ ID NO: 8 - DNA, 22 bp, synthetic construct
  source 1..22: mol_type = other DNA
acaggccgggacaagtgcaata